European Patent Application EP 4 382 536 A2, published June 12, 2024. Title: Anti-GM2AP ANTIBODY AND APPLICATIONS THEREOF. Applicant: Vitae Biomedical Co., Ltd. The sequence listing filed with the application follows.

SEQUENCE LISTING (33 sequences)

SEQ ID NO: 1 - protein, 193 aa, Homo sapiens
MQSLMQAPLLIALGLLLAAPAQAHLKKPSQLSSFSWDNCDEGKDPAVIRSLTLEPDPIIVPGNVTLSVMGSTSVPLSSPLKVDLVLEKEVAGLWIKIPCTDYIGSCTFEHFCDVLDMLIPTGEPCPEPLRTYGLPCHCPFKEGTYSLPKSEFVVPDLELPSWLTTGNYRIESVLSSSGKRLGCIKIAASLKGI

SEQ ID NO: 2 - protein, 193 aa, Homo sapiens [sequence omitted]

SEQ ID NO: 3 - protein, 202 aa, Homo sapiens
MQSLMQAPLLIALGLLLAAPAQAHLKKPSQLSSFSWDNCDEGKDPAVIRSLTLEPDPIIVPGNVTLSVMGSTSVPLSSPLKVDLVLEKEVAGLWIKIPCTDYIGSCTFEHFCDVLDMLIPTGEPCPEPLRTYGLPCHCPFKEGTYSLPKSEFVVPDLELPSWLTTGNYRIESVLSSSGKRLGCIKIAASLKGIRHHHHHHHH

SEQ ID NO: 4 - protein, 110 aa, synthetic construct
DIVMTQTASSVYVTPGESVSISCRSTKSLLHSNGDTYLYWFLQRPGQSPQLLIYRMSNLAPGVPDRFSGGGSGTAFTLRISRVEAEDVGVYYCMQHLEYPFTFGAGTKLE

SEQ ID NO: 5 - protein, 120 aa, synthetic construct
EIQLQQSGAELVRPGTSVKISCMASGYSFTGYNMNWVRQSHGRSLEWIGNINPYFGSPNYNQKFKGKATLTLDRSSNTAYMQLNRVTSEDSAVYYCASRQLGLGDTMDYWGQGTSVTVSS

SEQ ID NO: 6 - protein, 105 aa, synthetic construct
DIVMTQSHKFMSTSVGDRVTITCKASQDVSTAVGWYQQKPGQSPKLLIYWASTRHTGVPDRFTGSRFGTDYTLTISSVQAEDLALYYCQQHYITPWTFGGGTKLE

SEQ ID NO: 7 - protein, 119 aa, synthetic construct
QVQLQQPGADFVKPGASVKLSCKASGYTFTSYWINWVKQRPGQGLEWIGNIYPGSGSTNYNEKFKNKATLTIDTSSSTAYMQLSSLTSDDSAVYYCSRSTLYSYDDGSWGQGTTLTVSS

SEQ ID NO: 8 - protein, 105 aa, synthetic construct
DIQMTQSPSSLSASLGERVSLTCRASQEISGDLSWLQQKPDGTIKRLIYAASTLASGVPKRFSGSRSGSDYSLTISGLESEDFADYYCLQYVSYPFTFGSGTKLE

SEQ ID NO: 9 - protein, 117 aa, synthetic construct
QIQLQQSGPELGKPGASVKISCKASDYTFTDFYISWVKQRPGQGLEWIGWIYPLDDHTKYNEKFKGKATLTVDISSNTVYMQLSSLTSEDSAVYFCARIYGYAMDYWGQGTSVTVSS

SEQ ID NO: 10 - DNA, 330 bp, synthetic construct
  source 1..330: mol_type = other DNA
gatattgtgatgacccagaccgcttcctccgtgtatgtgacccctggcgagtccgtgtccatttcctgccgctccaccaagtccctgctgcactccaacggcgacacctacctgtattggttcctgcagaggccaggccagtctccccagctgctgatctacaggatgagcaatctggcaccaggagtgcctgacagattcagcggaggaggatccggaaccgcctttacactgcggatctctagagtggaggccgaggatgtgggcgtgtactattgtatgcagcacctggagtatccttttacctttggagccgggactaaactggaa

SEQ ID NO: 11 - DNA, 360 bp, synthetic construct
  source 1..360: mol_type = other DNA
gagatccagctgcagcagtctggagcagagctggtgcggccaggcacctctgtgaagatcagctgcatggcctccggctactctttcacaggctataacatgaattgggtgcggcagtcccacggcagatctctggagtggatcggcaacatcaatccctacttcggctcccctaactataatcagaagtttaagggcaaggccaccctgacactggacaggagctccaacaccgcctacatgcagctgaatcgcgtgacaagcgaggattccgccgtgtactattgtgcaagcaggcagctgggactgggcgacaccatggattattggggccagggcacctccgtgacagtgtctagc

SEQ ID NO: 12 - DNA, 315 bp, synthetic construct
  source 1..315: mol_type = other DNA
gacatcgtgatgacccagtctcacaagttcatgtctacaagcgtgggcgacagggtgaccatcacatgcaaggcatcccaggacgtgagcaccgcagtgggatggtaccagcagaagccaggccagagccctaagctgctgatctattgggcatccaccaggcacacaggcgtgccagacagattcaccggctccagatttggcacagattacaccctgacaatcagctccgtgcaggccgaggatctggccctgtactattgtcagcagcactatatcaccccctggacatttggcggcggcacaaagctggag

SEQ ID NO: 13 - DNA, 357 bp, synthetic construct
  source 1..357: mol_type = other DNA
caggtgcagctgcagcagccaggagcagacttcgtgaagcctggagcctccgtgaagctgtcttgcaaggccagcggctacacctttacaagctattggatcaactgggtgaagcagaggccaggacagggactggagtggatcggcaatatctaccccggctccggctctaccaactataatgagaagttcaagaacaaggccaccctgacaatcgataccagctcctctacagcctacatgcagctgagctccctgacctctgacgatagcgccgtgtactattgtagcagatccacactgtactcctatgacgatggctcttggggccagggcaccacactgacagtgtctagc

SEQ ID NO: 14 - DNA, 315 bp, synthetic construct
  source 1..315: mol_type = other DNA
gacatccagatgacccagagcccaagctccctgtctgccagcctgggagagagggtgtccctgacatgcagggcatctcaggagatcagcggcgacctgtcctggctgcagcagaagcccgatggcaccatcaagcggctgatctacgcagcatctacactggcaagcggagtgcctaagcggttctccggctctagaagcggctccgattattccctgaccatctctggcctggagagcgaggactttgccgattactattgtctgcagtacgtgtcctatcccttcacctttggctctggcacaaagctggag

SEQ ID NO: 15 - DNA, 351 bp, synthetic construct
  source 1..351: mol_type = other DNA
cagatccagctgcagcagtctggaccagagctgggcaagcctggagcctctgtgaagatcagctgcaaggcctccgactacaccttcacagacttctacatcagctgggtgaagcagaggccaggacagggactggagtggatcggctggatctaccccctggacgatcacaccaagtataacgagaagttcaagggcaaggccaccctgacagtggacatcagctccaataccgtgtacatgcagctgtctagcctgacaagcgaggactccgccgtgtacttttgtgccagaatctacggctatgccatggattattggggccagggcacctccgtgacagtgtcctct

SEQ ID NO: 16 - protein, 11 aa, synthetic construct
KSLLHSNGDTY

SEQ ID NO: 17 - skipped

SEQ ID NO: 18 - protein, 9 aa, synthetic construct
MQHLEYPFT

SEQ ID NO: 19 - protein, 8 aa, synthetic construct
GYSFTGYN

SEQ ID NO: 20 - protein, 8 aa, synthetic construct
INPYFGSP

SEQ ID NO: 21 - protein, 13 aa, synthetic construct
ASRQLGLGDTMDY

SEQ ID NO: 22 - protein, 6 aa, synthetic construct
QDVSTA

SEQ ID NO: 23 - skipped

SEQ ID NO: 24 - protein, 10 aa, synthetic construct
QQHYITPWTF

SEQ ID NO: 25 - protein, 8 aa, synthetic construct
GYTFTSYW

SEQ ID NO: 26 - protein, 8 aa, synthetic construct
IYPGSGST

SEQ ID NO: 27 - protein, 12 aa, synthetic construct
SRSTLYSYDDGS

SEQ ID NO: 28 - protein, 6 aa, synthetic construct
QEISGD

SEQ ID NO: 29 - skipped

SEQ ID NO: 30 - protein, 9 aa, synthetic construct
LQYVSYPFT

SEQ ID NO: 31 - protein, 8 aa, synthetic construct
DYTFTDFY

SEQ ID NO: 32 - protein, 8 aa, synthetic construct
IYPLDDHT

SEQ ID NO: 33 - protein, 10 aa, synthetic construct
ARIYGYAMDY